European Patent Application EP 4 338 585 A1, published March 20, 2024. Title: SPINACH PLANT COMPRISING A NOVEL LOCUS FOR DOWNY MILDEW RESISTANCE. Applicant: Sakata Seed Corporation. The sequence listing filed with the application follows.

SEQUENCE LISTING (27 sequences)

SEQ ID NO: 1 - DNA, 42 bp, Artificial Sequence
  Description of Artificial Sequence: Synthesized allele specific primer_1 for chr4_7421480.
gaaggtgaccaagttcatgctatccccggctttcttatcctg

SEQ ID NO: 2 - DNA, 42 bp, Artificial Sequence
  Description of Artificial Sequence: Synthesized allele specific primer_2 for chr4_7421480.
gaaggtcggagtcaacggattatccccggctttcttatcctc

SEQ ID NO: 3 - DNA, 21 bp, Artificial Sequence
  Description of Artificial Sequence: Synthesized common primer for chr4_7421480.
catgtgaaggaagggacacca

SEQ ID NO: 4 - DNA, 41 bp, Artificial Sequence
  Description of Artificial Sequence: Synthesized allele specific primer_1 for chr4_7962907.
gaaggtgaccaagttcatgctatgctcgtatacgcaatggc

SEQ ID NO: 5 - DNA, 42 bp, Artificial Sequence
  Description of Artificial Sequence: Synthesized allele specific primer_2 for chr4_7962907.
gaaggtcggagtcaacggattcatgctcgtatacgcaatggt

SEQ ID NO: 6 - DNA, 22 bp, Artificial Sequence
  Description of Artificial Sequence: Synthesized common primer for chr4_7962907.
ccaattgaccagaattgtcacc

SEQ ID NO: 7 - DNA, 43 bp, Artificial Sequence
  Description of Artificial Sequence: Synthesized allele specific primer_1 for chr4_8152986.
gaaggtgaccaagttcatgctgggagcaacatttatgcaagac

SEQ ID NO: 8 - DNA, 43 bp, Artificial Sequence
  Description of Artificial Sequence: Synthesized allele specific primer_2 for chr4_8152986.
gaaggtcggagtcaacggattgggagcaacatttatgcaagat

SEQ ID NO: 9 - DNA, 21 bp, Artificial Sequence
  Description of Artificial Sequence: Synthesized common primer for chr4_8152986.
atgtatggtctgacaacggca

SEQ ID NO: 10 - DNA, 42 bp, Artificial Sequence
  Description of Artificial Sequence: Synthesized allele specific primer_1 for chr4_8190990.
gaaggtgaccaagttcatgctatcgggaggaaagctctaacc

SEQ ID NO: 11 - DNA, 42 bp, Artificial Sequence
  Description of Artificial Sequence: Synthesized allele specific primer_2 for chr4_8190990.
gaaggtcggagtcaacggattatcgggaggaaagctctaact

SEQ ID NO: 12 - DNA, 21 bp, Artificial Sequence
  Description of Artificial Sequence: Synthesized common primer for chr4_8190990.
tgtgtacccatattggccaga

SEQ ID NO: 13 - DNA, 41 bp, Artificial Sequence
  Description of Artificial Sequence: Synthesized allele specific primer_1 for chr4_8488603.
gaaggtcggagtcaacggatttaatgggatctgctgcctcg

SEQ ID NO: 14 - DNA, 42 bp, Artificial Sequence
  Description of Artificial Sequence: Synthesized allele specific primer_2 for chr4_8488603.
gaaggtgaccaagttcatgctctaatgggatctgctgcctca

SEQ ID NO: 15 - DNA, 21 bp, Artificial Sequence
  Description of Artificial Sequence: Synthesized common primer for chr4_8488603.
caaaggcttgacggtccagta

SEQ ID NO: 16 - DNA, 42 bp, Artificial Sequence
  Description of Artificial Sequence: Synthesized allele specific primer_1 for chr4_8494600.
gaaggtgaccaagttcatgcttctcgcttgtcattgtcagca

SEQ ID NO: 17 - DNA, 41 bp, Artificial Sequence
  Description of Artificial Sequence: Synthesized allele specific primer_2 for chr4_8494600.
gaaggtcggagtcaacggattttcgcttgtcattgtcagcg

SEQ ID NO: 18 - DNA, 21 bp, Artificial Sequence
  Description of Artificial Sequence: Synthesized common primer for chr4_8494600.
ctgtggagtcggaagaacaca

SEQ ID NO: 19 - DNA, 44 bp, Artificial Sequence
  Description of Artificial Sequence: Synthesized allele specific primer_1 for chr4_8510715.
gaaggtgaccaagttcatgctctggtccatactcatactcaggg

SEQ ID NO: 20 - DNA, 44 bp, Artificial Sequence
  Description of Artificial Sequence: Synthesized allele specific primer_2 for chr4_8510715.
gaaggtcggagtcaacggattctggtccatactcatactcaggc

SEQ ID NO: 21 - DNA, 21 bp, Artificial Sequence
  Description of Artificial Sequence: Synthesized common primer for chr4_8510715.
agctaattctgagccaaggcc

SEQ ID NO: 22 - DNA, 45 bp, Artificial Sequence
  Description of Artificial Sequence: Synthesized allele specific primer_1 for chr4_8617232.
gaaggtcggagtcaacggatttgagacagcgggataaagagtaag

SEQ ID NO: 23 - DNA, 45 bp, Artificial Sequence
  Description of Artificial Sequence: Synthesized allele specific primer_2 for chr4_8617232.
gaaggtgaccaagttcatgcttgagacagcgggataaagagtaaa

SEQ ID NO: 24 - DNA, 21 bp, Artificial Sequence
  Description of Artificial Sequence: Synthesized common primer for chr4_8617232.
tcagttcgacaagctgcctag

SEQ ID NO: 25 - DNA, 40 bp, Artificial Sequence
  Description of Artificial Sequence: Synthesized allele specific primer_1 for chr4_10710358.
gaaggtcggagtcaacggattcgagttgatcacctcgtcg

SEQ ID NO: 26 - DNA, 40 bp, Artificial Sequence
  Description of Artificial Sequence: Synthesized allele specific primer_2 for chr4_10710358.
gaaggtgaccaagttcatgctcgagttgatcacctcgtcc

SEQ ID NO: 27 - DNA, 19 bp, Artificial Sequence
  Description of Artificial Sequence: Synthesized common primer for chr4_10710358.
tgtacccagttgtcgagcc